European Patent Application EP 4 628 892 A1, published October 8, 2025. Title: Inhibitor of activity or expression of NgR1 protein for improving cytolytic activity by promoting formation of immunological synapse of immune cells. Applicant: Korea Research Institute of Bioscience and Biotechnology. Application KR. The sequence listing filed with the application follows.

SEQUENCE LISTING (111 sequences)

SEQ ID NO: 1 - protein, 8 aa, synthetic construct
GFNFNDYA

SEQ ID NO: 2 - DNA, 24 bp, synthetic construct
  source 1..24: mol_type = other DNA
ggattcaactttaatgattatgcc

SEQ ID NO: 3 - protein, 8 aa, synthetic construct
ISWNSGAI

SEQ ID NO: 4 - DNA, 24 bp, synthetic construct
  source 1..24: mol_type = other DNA
attagttggaatagtggtgccata

SEQ ID NO: 5 - protein, 17 aa, synthetic construct
ARDYYYETSGYYYGFDN

SEQ ID NO: 6 - DNA, 51 bp, synthetic construct
  source 1..51: mol_type = other DNA
gcgagagattactactatgagaccagtggttactattatgggtttgacaac

SEQ ID NO: 7 - protein, 17 aa, synthetic construct
ARDYNYEISGYYYGFDN

SEQ ID NO: 8 - DNA, 51 bp, synthetic construct
  source 1..51: mol_type = other DNA
gcgagagattacaactatgagatcagtggttactattatgggtttgacaac

SEQ ID NO: 9 - protein, 17 aa, synthetic construct
ARDYNYETSGYYHGFDN

SEQ ID NO: 10 - DNA, 51 bp, synthetic construct
  source 1..51: mol_type = other DNA
gcgagagattacaactatgagaccagtggttactatcatgggtttgacaac

SEQ ID NO: 11 - protein, 124 aa, synthetic construct
QMQLVQSGGGLEQPGRSLRLSCVTSGFNFNDYAMHWVRQAPGKGLEWVSGISWNSGAIGYADSVKGRFTVSRDNSKNSLYLQMNSLRAEDTAVYYCARDYYYETSGYYYGFDNWGQGTLVTVSS

SEQ ID NO: 12 - DNA, 372 bp, synthetic construct
  source 1..372: mol_type = other DNA
cagatgcagctggtgcagtctgggggaggcttggaacagcctggcaggtccctgagactctcctgtgtaacctctggattcaactttaatgattatgccatgcactgggtccggcaagctccagggaagggcctggagtgggtctcaggtattagttggaatagtggtgccataggctatgcggactctgtgaagggccgattcaccgtctccagagacaacagcaaaaactccctgtatctgcaaatgaacagtctgagagccgaggacacggccgtgtattactgtgcgagagattactactatgagaccagtggttactattatgggtttgacaactggggccagggaaccctggtcaccgtctcctca

SEQ ID NO: 13 - protein, 124 aa, synthetic construct
QMQLVQSGGGLEQPGRSLRLSCVTSGFNFNDYAMHWVRQAPGKGLEWVSGISWNSGAIGYADSVKGRFTVSRDNSKNSLYLQMNSLRAEDTAVYYCARDYNYEISGYYYGFDNWGQGTLVTVSS

SEQ ID NO: 14 - DNA, 372 bp, synthetic construct
  source 1..372: mol_type = other DNA
cagatgcagctggtgcagtctgggggaggcttggaacagcctggcaggtccctgagactctcctgtgtaacctctggattcaactttaatgattatgccatgcactgggtccggcaagctccagggaagggcctggagtgggtctcaggtattagttggaatagtggtgccataggctatgcggactctgtgaagggccgattcaccgtctccagagacaacagcaaaaactccctgtatctgcaaatgaacagtctgagagccgaggacacggccgtgtattactgtgcgagagattacaactatgagatcagtggttactattatgggtttgacaactggggccagggaaccctggtcaccgtctcctca

SEQ ID NO: 15 - protein, 124 aa, synthetic construct
QMQLVQSGGGLEQPGRSLRLSCVTSGFNFNDYAMHWVRQAPGKGLEWVSGISWNSGAIGYADSVKGRFTVSRDNSKNSLYLQMNSLRAEDTAVYYCARDYNYETSGYYHGFDNWGQGTLVTVSS

SEQ ID NO: 16 - DNA, 372 bp, synthetic construct
  source 1..372: mol_type = other DNA
cagatgcagctggtgcagtctgggggaggcttggaacagcccggcaggtccctgagactctcctgtgtaacctctggattcaactttaatgattatgccatgcactgggtccggcaagctccagggaagggcctggagtgggtctcaggtattagttggaatagtggtgccataggctatgcggactctgtgaagggccgattcaccgtctccagagacaacagcaaaaactccctgtatctgcaaatgaacagtctgagagccgaggacacggccgtgtattactgtgcgagagattacaactatgagaccagtggttactatcatgggtttgacaactggggccagggaaccctggtcaccgtctcctca

SEQ ID NO: 17 - protein, 454 aa, synthetic construct
QMQLVQSGGGLEQPGRSLRLSCVTSGFNFNDYAMHWVRQAPGKGLEWVSGISWNSGAIGYADSVKGRFTVSRDNSKNSLYLQMNSLRAEDTAVYYCARDYYYETSGYYYGFDNWGQGTLVTVSSASTKGPSVFPLAPSSKSTSGGTAALGCLVKDYFPEPVTVSWNSGALTSGVHTFPAVLQSSGLYSLSSVVTVPSSSLGTQTYICNVNHKPSNTKVDKKVEPKSCDKTHTCPPCPAPELLGGPSVFLFPPKPKDTLMISRTPEVTCVVVDVSHEDPEVKFNWYVDGVEVHNAKTKPREEQYNSTYRVVSVLTVLHQDWLNGKEYKCKVSNKALPAPIEKTISKAKGQPREPQVYTLPPSREEMTKNQVSLTCLVKGFYPSDIAVEWESNGQPENNYKTTPPVLDSDGSFFLYSKLTVDKSRWQQGNVFSCSVMHEALHNHYTQKSLSLSPGK

SEQ ID NO: 18 - DNA, 1362 bp, synthetic construct
  source 1..1362: mol_type = other DNA
cagatgcagctggtgcagtctgggggaggcttggaacagcctggcaggtccctgagactctcctgtgtaacctctggattcaactttaatgattatgccatgcactgggtccggcaagctccagggaagggcctggagtgggtctcaggtattagttggaatagtggtgccataggctatgcggactctgtgaagggccgattcaccgtctccagagacaacagcaaaaactccctgtatctgcaaatgaacagtctgagagccgaggacacggccgtgtattactgtgcgagagattactactatgagaccagtggttactattatgggtttgacaactggggccagggaaccctggtcaccgtctcctcagctagcaccaagggcccatcggtcttccccctggcgccctcctccaagagcacctctgggggcacagcggccctgggctgcctggtcaaggactacttccccgaaccggtgacggtgtcgtggaactcaggggccctgaccagcggcgtgcacaccttcccggctgtcctacagtcctcaggactctactccctcagcagcgtggtgaccgtgccctccagcagcctgggcacccagacctacatctgcaacgtgaatcacaagcccagcaacaccaaggtggacaagaaagttgagcccaaatcttgtgacaaaactcacacatgcccaccgtgcccagcacctgaactcctggggggaccgtcagtcttcctcttccccccaaaacccaaggacaccctcatgatctcccggacccctgaggtcacatgcgtggtggtggacgtgagccacgaagaccctgaggtcaagttcaactggtacgtggacggcgtggaggtgcataatgccaagacaaagccgcgggaggagcagtacaacagcacgtaccgtgtggtcagcgtcctcaccgtcctgcaccaggactggctgaatggcaaggagtacaagtgcaaggtctccaacaaagccctcccagcccccatcgagaaaaccatctccaaagccaaagggcagccccgagaaccacaggtgtacaccctgcccccatcccgggaggagatgaccaagaaccaggtcagcctgacctgcctggtcaaaggcttctatcccagcgacatcgccgtggagtgggagagcaatgggcagccggagaacaactacaagaccacgcctcccgtgctggactccgacggctccttcttcctctacagcaagctcaccgtggacaagagcaggtggcagcaggggaacgtcttctcatgctccgtgatgcatgaggctctgcacaaccactacacgcagaagagcctctccctgtctccgggtaaa

SEQ ID NO: 19 - protein, 454 aa, synthetic construct
QMQLVQSGGGLEQPGRSLRLSCVTSGFNFNDYAMHWVRQAPGKGLEWVSGISWNSGAIGYADSVKGRFTVSRDNSKNSLYLQMNSLRAEDTAVYYCARDYNYEISGYYYGFDNWGQGTLVTVSSASTKGPSVFPLAPSSKSTSGGTAALGCLVKDYFPEPVTVSWNSGALTSGVHTFPAVLQSSGLYSLSSVVTVPSSSLGTQTYICNVNHKPSNTKVDKKVEPKSCDKTHTCPPCPAPELLGGPSVFLFPPKPKDTLMISRTPEVTCVVVDVSHEDPEVKFNWYVDGVEVHNAKTKPREEQYNSTYRVVSVLTVLHQDWLNGKEYKCKVSNKALPAPIEKTISKAKGQPREPQVYTLPPSREEMTKNQVSLTCLVKGFYPSDIAVEWESNGQPENNYKTTPPVLDSDGSFFLYSKLTVDKSRWQQGNVFSCSVMHEALHNHYTQKSLSLSPGK

SEQ ID NO: 20 - DNA, 1362 bp, synthetic construct
  source 1..1362: mol_type = other DNA
cagatgcagctggtgcagtctgggggaggcttggaacagcctggcaggtccctgagactctcctgtgtaacctctggattcaactttaatgattatgccatgcactgggtccggcaagctccagggaagggcctggagtgggtctcaggtattagttggaatagtggtgccataggctatgcggactctgtgaagggccgattcaccgtctccagagacaacagcaaaaactccctgtatctgcaaatgaacagtctgagagccgaggacacggccgtgtattactgtgcgagagattacaactatgagatcagtggttactattatgggtttgacaactggggccagggaaccctggtcaccgtctcctcagctagcaccaagggcccatcggtcttccccctggcgccctcctccaagagcacctctgggggcacagcggccctgggctgcctggtcaaggactacttccccgaaccggtgacggtgtcgtggaactcaggggccctgaccagcggcgtgcacaccttcccggctgtcctacagtcctcaggactctactccctcagcagcgtggtgaccgtgccctccagcagcctgggcacccagacctacatctgcaacgtgaatcacaagcccagcaacaccaaggtggacaagaaagttgagcccaaatcttgtgacaaaactcacacatgcccaccgtgcccagcacctgaactcctggggggaccgtcagtcttcctcttccccccaaaacccaaggacaccctcatgatctcccggacccctgaggtcacatgcgtggtggtggacgtgagccacgaagaccctgaggtcaagttcaactggtacgtggacggcgtggaggtgcataatgccaagacaaagccgcgggaggagcagtacaacagcacgtaccgtgtggtcagcgtcctcaccgtcctgcaccaggactggctgaatggcaaggagtacaagtgcaaggtctccaacaaagccctcccagcccccatcgagaaaaccatctccaaagccaaagggcagccccgagaaccacaggtgtacaccctgcccccatcccgggaggagatgaccaagaaccaggtcagcctgacctgcctggtcaaaggcttctatcccagcgacatcgccgtggagtgggagagcaatgggcagccggagaacaactacaagaccacgcctcccgtgctggactccgacggctccttcttcctctacagcaagctcaccgtggacaagagcaggtggcagcaggggaacgtcttctcatgctccgtgatgcatgaggctctgcacaaccactacacgcagaagagcctctccctgtctccgggtaaa

SEQ ID NO: 21 - protein, 454 aa, synthetic construct
QMQLVQSGGGLEQPGRSLRLSCVTSGFNFNDYAMHWVRQAPGKGLEWVSGISWNSGAIGYADSVKGRFTVSRDNSKNSLYLQMNSLRAEDTAVYYCARDYNYETSGYYHGFDNWGQGTLVTVSSASTKGPSVFPLAPSSKSTSGGTAALGCLVKDYFPEPVTVSWNSGALTSGVHTFPAVLQSSGLYSLSSVVTVPSSSLGTQTYICNVNHKPSNTKVDKKVEPKSCDKTHTCPPCPAPELLGGPSVFLFPPKPKDTLMISRTPEVTCVVVDVSHEDPEVKFNWYVDGVEVHNAKTKPREEQYNSTYRVVSVLTVLHQDWLNGKEYKCKVSNKALPAPIEKTISKAKGQPREPQVYTLPPSREEMTKNQVSLTCLVKGFYPSDIAVEWESNGQPENNYKTTPPVLDSDGSFFLYSKLTVDKSRWQQGNVFSCSVMHEALHNHYTQKSLSLSPGK

SEQ ID NO: 22 - DNA, 1362 bp, synthetic construct
  source 1..1362: mol_type = other DNA
cagatgcagctggtgcagtctgggggaggcttggaacagcccggcaggtccctgagactctcctgtgtaacctctggattcaactttaatgattatgccatgcactgggtccggcaagctccagggaagggcctggagtgggtctcaggtattagttggaatagtggtgccataggctatgcggactctgtgaagggccgattcaccgtctccagagacaacagcaaaaactccctgtatctgcaaatgaacagtctgagagccgaggacacggccgtgtattactgtgcgagagattacaactatgagaccagtggttactatcatgggtttgacaactggggccagggaaccctggtcaccgtctcctcagctagcaccaagggcccatcggtcttccccctggcgccctcctccaagagcacctctgggggcacagcggccctgggctgcctggtcaaggactacttccccgaaccggtgacggtgtcgtggaactcaggggccctgaccagcggcgtgcacaccttcccggctgtcctacagtcctcaggactctactccctcagcagcgtggtgaccgtgccctccagcagcctgggcacccagacctacatctgcaacgtgaatcacaagcccagcaacaccaaggtggacaagaaagttgagcccaaatcttgtgacaaaactcacacatgcccaccgtgcccagcacctgaactcctggggggaccgtcagtcttcctcttccccccaaaacccaaggacaccctcatgatctcccggacccctgaggtcacatgcgtggtggtggacgtgagccacgaagaccctgaggtcaagttcaactggtacgtggacggcgtggaggtgcataatgccaagacaaagccgcgggaggagcagtacaacagcacgtaccgtgtggtcagcgtcctcaccgtcctgcaccaggactggctgaatggcaaggagtacaagtgcaaggtctccaacaaagccctcccagcccccatcgagaaaaccatctccaaagccaaagggcagccccgagaaccacaggtgtacaccctgcccccatcccgggaggagatgaccaagaaccaggtcagcctgacctgcctggtcaaaggcttctatcccagcgacatcgccgtggagtgggagagcaatgggcagccggagaacaactacaagaccacgcctcccgtgctggactccgacggctccttcttcctctacagcaagctcaccgtggacaagagcaggtggcagcaggggaacgtcttctcatgctccgtgatgcatgaggctctgcacaaccactacacgcagaagagcctctccctgtctccgggtaaa

SEQ ID NO: 23 - protein, 6 aa, synthetic construct
QGISRW

SEQ ID NO: 24 - DNA, 18 bp, synthetic construct
  source 1..18: mol_type = other DNA
cagggtattagtaggtgg

SEQ ID NO: 25-26 - skipped (2 entries)

SEQ ID NO: 27 - protein, 9 aa, synthetic construct
QQTNNFPYT

SEQ ID NO: 28 - DNA, 27 bp, synthetic construct
  source 1..27: mol_type = other DNA
caacagactaacaatttcccgtacact

SEQ ID NO: 29 - protein, 108 aa, synthetic construct
DIQMTQSPSSVSASVGDRVTITCRASQGISRWLAWYQQKPGKAPKLLIYAASNLQSGVPLRFSGSGSGTDFTLTINSLQPEDSATYYCQQTNNFPYTFGQGTKVEIKR

SEQ ID NO: 30 - DNA, 324 bp, synthetic construct
  source 1..324: mol_type = other DNA
gacatccagatgacccagtctccatcttccgtgtctgcatctgtaggagacagagtcaccatcacttgtcgggcgagtcagggtattagtaggtggttagcctggtatcagcagaaaccagggaaagcccctaaactcctgatctatgctgcatccaatttgcaaagtggggtcccgttaagattcagcggcagtggatctgggacagatttcactctcactatcaacagcctgcagcctgaagattctgcaacttattactgtcaacagactaacaatttcccgtacacttttggccaagggaccaaggtggaaatcaaacgt

SEQ ID NO: 31 - protein, 108 aa, synthetic construct
DIQMTQSPSSVSASVGDRVTITCRASQGISRWLSWYQQKPGKAPKLLIYAASNLQSGVPLRFSGSGFGTDFTLTINSLQPEDSATYYCQQTNNFPYTFGQGTKVEIKR

SEQ ID NO: 32 - DNA, 324 bp, synthetic construct
  source 1..324: mol_type = other DNA
gacatccagatgacccagtctccatcttccgtgtctgcatctgtaggggacagagtcaccatcacttgtcgggcgagtcagggtattagtaggtggttatcctggtatcagcagaaaccagggaaagcccctaaactcctgatctatgctgcatccaatttgcaaagtggggtcccgttaagattcagcggcagtggatttgggacagatttcactctcactatcaacagcctgcagcctgaagattctgcaacttattactgtcaacagactaacaatttcccgtacacttttggccaagggaccaaggtggaaatcaaacgt

SEQ ID NO: 33 - protein, 108 aa, synthetic construct
DIQMTQSPSSVSASVGDRVTITCRASQGISRWLSWYQQKPGKAPKLLIYAASNLQSGVPLRFSGSGSGTDFTLTINSLQPEDSATYYCQQTNNFPYTFGQGTKVEIKR

SEQ ID NO: 34 - DNA, 324 bp, synthetic construct
  source 1..324: mol_type = other DNA
gacatccagatgacccagtctccatcttccgtgtctgcatctgtaggggacagagtcaccatcacttgtcgggcgagtcagggtattagtaggtggttatcctggtatcagcagaaaccagggaaagcccctaaactcctgatctatgctgcatccaatttgcaaagtggggtcccgttaagattcagcggcagtggatctgggacagatttcactctcactatcaacagcctgcagcctgaagattctgcaacttattactgtcaacagactaacaatttcccgtacacttttggccaagggaccaaggtggaaatcaaacgt

SEQ ID NO: 35 - protein, 214 aa, synthetic construct
DIQMTQSPSSVSASVGDRVTITCRASQGISRWLAWYQQKPGKAPKLLIYAASNLQSGVPLRFSGSGSGTDFTLTINSLQPEDSATYYCQQTNNFPYTFGQGTKVEIKRTVAAPSVFIFPPSDEQLKSGTASVVCLLNNFYPREAKVQWKVDNALQSGNSQESVTEQDSKDSTYSLSSTLTLSKADYEKHKVYACEVTHQGLSSPVTKSFNRGEC

SEQ ID NO: 36 - DNA, 642 bp, synthetic construct
  source 1..642: mol_type = other DNA
gacatccagatgacccagtctccatcttccgtgtctgcatctgtaggagacagagtcaccatcacttgtcgggcgagtcagggtattagtaggtggttagcctggtatcagcagaaaccagggaaagcccctaaactcctgatctatgctgcatccaatttgcaaagtggggtcccgttaagattcagcggcagtggatctgggacagatttcactctcactatcaacagcctgcagcctgaagattctgcaacttattactgtcaacagactaacaatttcccgtacacttttggccaagggaccaaggtggaaatcaaacgtacggtggctgcaccatctgtcttcatcttcccgccatctgatgagcagttgaaatctggaactgcctctgttgtgtgcctgctgaataacttctatcccagagaggccaaagtacagtggaaggtggataacgccctccaatcgggtaactcccaggagagtgtcacagagcaggacagcaaggacagcacctacagcctcagcagcaccctgacgctgagcaaagcagactacgagaaacacaaagtctacgcctgcgaagtcacccatcagggcctgagctcgcccgtcacaaagagcttcaacaggggagagtgt

SEQ ID NO: 37 - protein, 214 aa, synthetic construct
DIQMTQSPSSVSASVGDRVTITCRASQGISRWLSWYQQKPGKAPKLLIYAASNLQSGVPLRFSGSGFGTDFTLTINSLQPEDSATYYCQQTNNFPYTFGQGTKVEIKRTVAAPSVFIFPPSDEQLKSGTASVVCLLNNFYPREAKVQWKVDNALQSGNSQESVTEQDSKDSTYSLSSTLTLSKADYEKHKVYACEVTHQGLSSPVTKSFNRGEC

SEQ ID NO: 38 - DNA, 642 bp, synthetic construct
  source 1..642: mol_type = other DNA
gacatccagatgacccagtctccatcttccgtgtctgcatctgtaggggacagagtcaccatcacttgtcgggcgagtcagggtattagtaggtggttatcctggtatcagcagaaaccagggaaagcccctaaactcctgatctatgctgcatccaatttgcaaagtggggtcccgttaagattcagcggcagtggatttgggacagatttcactctcactatcaacagcctgcagcctgaagattctgcaacttattactgtcaacagactaacaatttcccgtacacttttggccaagggaccaaggtggaaatcaaacgtacggtggctgcaccatctgtcttcatcttcccgccatctgatgagcagttgaaatctggaactgcctctgttgtgtgcctgctgaataacttctatcccagagaggccaaagtacagtggaaggtggataacgccctccaatcgggtaactcccaggagagtgtcacagagcaggacagcaaggacagcacctacagcctcagcagcaccctgacgctgagcaaagcagactacgagaaacacaaagtctacgcctgcgaagtcacccatcagggcctgagctcgcccgtcacaaagagcttcaacaggggagagtgt

SEQ ID NO: 39 - protein, 214 aa, synthetic construct
DIQMTQSPSSVSASVGDRVTITCRASQGISRWLSWYQQKPGKAPKLLIYAASNLQSGVPLRFSGSGSGTDFTLTINSLQPEDSATYYCQQTNNFPYTFGQGTKVEIKRTVAAPSVFIFPPSDEQLKSGTASVVCLLNNFYPREAKVQWKVDNALQSGNSQESVTEQDSKDSTYSLSSTLTLSKADYEKHKVYACEVTHQGLSSPVTKSFNRGEC

SEQ ID NO: 40 - DNA, 642 bp, synthetic construct
  source 1..642: mol_type = other DNA
gacatccagatgacccagtctccatcttccgtgtctgcatctgtaggggacagagtcaccatcacttgtcgggcgagtcagggtattagtaggtggttatcctggtatcagcagaaaccagggaaagcccctaaactcctgatctatgctgcatccaatttgcaaagtggggtcccgttaagattcagcggcagtggatctgggacagatttcactctcactatcaacagcctgcagcctgaagattctgcaacttattactgtcaacagactaacaatttcccgtacacttttggccaagggaccaaggtggaaatcaaacgtacggtggctgcaccatctgtcttcatcttcccgccatctgatgagcagttgaaatctggaactgcctctgttgtgtgcctgctgaataacttctatcccagagaggccaaagtacagtggaaggtggataacgccctccaatcgggtaactcccaggagagtgtcacagagcaggacagcaaggacagcacctacagcctcagcagcaccctgacgctgagcaaagcagactacgagaaacacaaagtctacgcctgcgaagtcacccatcagggcctgagctcgcccgtcacaaagagcttcaacaggggagagtgt

SEQ ID NO: 41 - protein, 8 aa, synthetic construct
GYTLSELS

SEQ ID NO: 42 - DNA, 24 bp, synthetic construct
  source 1..24: mol_type = other DNA
ggttacacccttagtgagttatcc

SEQ ID NO: 43 - protein, 8 aa, synthetic construct
GYPLSELS

SEQ ID NO: 44 - DNA, 24 bp, synthetic construct
  source 1..24: mol_type = other DNA
ggttacccccttagtgagttatcc

SEQ ID NO: 45 - protein, 8 aa, synthetic construct
GYTLSGLS

SEQ ID NO: 46 - DNA, 24 bp, synthetic construct
  source 1..24: mol_type = other DNA
ggttacacccttagtgggttatcc

SEQ ID NO: 47 - protein, 8 aa, synthetic construct
FDPEDDET

SEQ ID NO: 48 - DNA, 24 bp, synthetic construct
  source 1..24: mol_type = other DNA
tttgatcctgaagatgatgaaaca

SEQ ID NO: 49 - protein, 8 aa, synthetic construct
FDSEDDET

SEQ ID NO: 50 - DNA, 24 bp, synthetic construct
  source 1..24: mol_type = other DNA
tttgattctgaagatgatgaaaca

SEQ ID NO: 51 - protein, 18 aa, synthetic construct
ARDLGYLTSGNYYDAFDI

SEQ ID NO: 52 - DNA, 54 bp, synthetic construct
  source 1..54: mol_type = other DNA
gcgagggatctgggttaccttacttcggggaattattatgatgcttttgatatc

SEQ ID NO: 53 - protein, 18 aa, synthetic construct
ARDLGYLTSGNYYDAFGI

SEQ ID NO: 54 - DNA, 54 bp, synthetic construct
  source 1..54: mol_type = other DNA
gcgagggatctgggttaccttacttcggggaattattatgatgcttttggtatc

SEQ ID NO: 55 - protein, 18 aa, synthetic construct
ARDLGYLTSGNYYNAFGI

SEQ ID NO: 56 - DNA, 54 bp, synthetic construct
  source 1..54: mol_type = other DNA
gcgagggatctgggttaccttacttcggggaattattataatgcttttggtatc

SEQ ID NO: 57 - protein, 18 aa, synthetic construct
ARDLGYLTSGNYYDAFDF

SEQ ID NO: 58 - DNA, 54 bp, synthetic construct
  source 1..54: mol_type = other DNA
gcgagggatctgggttaccttacttcggggaattattatgatgcttttgatttc

SEQ ID NO: 59 - protein, 125 aa, synthetic construct
QMQLVQSGAEVKKPGASVKVSCKVSGYTLSELSIHWVRQAPGKGLEWMGGFDPEDDETVYAQKFQGRVTLTDDTSTDTAYMELSSLRSEDTAVYYCARDLGYLTSGNYYDAFDIWGRGTMITVSS

SEQ ID NO: 60 - DNA, 375 bp, synthetic construct
  source 1..375: mol_type = other DNA
cagatgcagctggtacagtctggggctgaggtgaagaagcctggggcctcagtgaaggtctcctgcaaagtttccggttacacccttagtgagttatccattcactgggtgcgacaggctcctggaaaagggcttgagtggatggggggttttgatcctgaagatgatgaaacagtctacgcacagaagttccagggcagagtcaccttgaccgacgacacatctacagacacagcctacatggagctgagcagcctgagatctgaggacacggccgtgtattactgtgcgagggatctgggttaccttacttcggggaattattatgatgcttttgatatctggggccgagggacaatgatcaccgtctcctca

SEQ ID NO: 61 - protein, 125 aa, synthetic construct
QMQLVQSGAEVKKPGASVKVSCKVSGYPLSELSIHWVRQAPGKGLEWMGGFDSEDDETVYAQKFQGRVTLTDDTSTDTAYMELSSLRSEDTAVYYCARDLGYLTSGNYYDAFGIWGRGTMITVSS

SEQ ID NO: 62 - DNA, 375 bp, synthetic construct
  source 1..375: mol_type = other DNA
cagatgcagctggtacagtctggggctgaggtgaagaagcctggggcctcagtgaaggtctcctgcaaagtttccggttacccccttagtgagttatccattcactgggtgcgacaggctcctggaaaagggcttgagtggatggggggttttgattctgaagatgatgaaacagtctacgcacagaagttccagggcagagtcaccttgaccgacgacacatctacagacacagcctacatggagctgagcagcctgagatctgaggacacggccgtgtattactgtgcgagggatctgggttaccttacttcggggaattattatgatgcttttggtatctggggccgagggacaatgatcaccgtctcctca

SEQ ID NO: 63 - protein, 125 aa, synthetic construct
QMQLVQSGAEVKKPGASVKVSCKVSGYTLSELSIHWVRQAPGKGLEWMGGFDPEDDETVYAQKFQGRVTLTDDTSTDTAYMELSSLRSEDTAVYYCARDLGYLTSGNYYNAFGIWGRGTMITVSS

SEQ ID NO: 64 - DNA, 375 bp, synthetic construct
  source 1..375: mol_type = other DNA
cagatgcagctggtacagtctggggctgaggtgaagaagcctggggcctcagtgaaggtctcctgcaaagtttccggttacacccttagtgagttatccattcactgggtgcgacaggctcctggaaaagggcttgagtggatggggggttttgatcctgaagatgatgaaacagtctacgcacagaagttccagggcagagtcaccttgaccgacgacacatctacagacacagcctacatggagctgagcagcctgagatctgaggacacggccgtgtattactgtgcgagggatctgggttaccttacttcggggaattattataatgcttttggtatctggggccgagggacaatgatcaccgtctcctca

SEQ ID NO: 65 - protein, 125 aa, synthetic construct
QMQLVQSGAEVKKPGASVKVSCKVSGYTLSGLSIHWVRQAPGKGLEWMGGFDSEDDETVYAQKFQGRVTLTDDTSTDTAYMELSSLRSEDTAVYYCARDLGYLTSGNYYDAFDIWGRGTMITVSS

SEQ ID NO: 66 - DNA, 375 bp, synthetic construct
  source 1..375: mol_type = other DNA
cagatgcagctggtacagtctggggctgaggtgaagaagcctggggcctcagtgaaggtctcctgcaaagtttccggttacacccttagtgggttatccattcactgggtgcgacaggctcctggaaaagggcttgagtggatggggggttttgattctgaagatgatgaaacagtctacgcacagaagttccagggcagagtcaccttgaccgacgacacatctacagacacagcctacatggagctgagcagcctgagatctgaggacacggccgtgtattactgtgcgagggatctgggttaccttacttcggggaattattatgatgcttttgatatctggggccgagggacaatgatcaccgtctcctca

SEQ ID NO: 67 - protein, 125 aa, synthetic construct
QMQLVQSGAEVKKPGASVKVSCKVSGYTLSELSIHWVRQAPGKGLEWMGGFDSEDDETVYAQKFQGRVTLTDDTSTDTAYMELSSLRSEDTAVYYCARDLGYLTSGNYYDAFDFWGRGTMITVSS

SEQ ID NO: 68 - DNA, 375 bp, synthetic construct
  source 1..375: mol_type = other DNA
cagatgcagctggtacagtctggggctgaggtgaagaagcctggggcctcagtgaaggtctcctgcaaagtttccggttacacccttagtgagttatccattcactgggtgcgacaggctcctggaaaagggcttgagtggatggggggttttgattctgaagatgatgaaacagtctacgcacagaagttccagggcagagtcaccttgaccgacgacacatctacagacacagcctacatggagctgagcagcctgagatctgaggacacggccgtgtattactgtgcgagggatctgggttaccttacttcggggaattattatgatgcttttgatttctggggccgagggacaatgatcaccgtctcctca

SEQ ID NO: 69 - protein, 455 aa, synthetic construct
QMQLVQSGAEVKKPGASVKVSCKVSGYTLSELSIHWVRQAPGKGLEWMGGFDPEDDETVYAQKFQGRVTLTDDTSTDTAYMELSSLRSEDTAVYYCARDLGYLTSGNYYDAFDIWGRGTMITVSSASTKGPSVFPLAPSSKSTSGGTAALGCLVKDYFPEPVTVSWNSGALTSGVHTFPAVLQSSGLYSLSSVVTVPSSSLGTQTYICNVNHKPSNTKVDKKVEPKSCDKTHTCPPCPAPELLGGPSVFLFPPKPKDTLMISRTPEVTCVVVDVSHEDPEVKFNWYVDGVEVHNAKTKPREEQYNSTYRVVSVLTVLHQDWLNGKEYKCKVSNKALPAPIEKTISKAKGQPREPQVYTLPPSREEMTKNQVSLTCLVKGFYPSDIAVEWESNGQPENNYKTTPPVLDSDGSFFLYSKLTVDKSRWQQGNVFSCSVMHEALHNHYTQKSLSLSPGK

SEQ ID NO: 70 - DNA, 1365 bp, synthetic construct
  source 1..1365: mol_type = other DNA
cagatgcagctggtacagtctggggctgaggtgaagaagcctggggcctcagtgaaggtctcctgcaaagtttccggttacacccttagtgagttatccattcactgggtgcgacaggctcctggaaaagggcttgagtggatggggggttttgatcctgaagatgatgaaacagtctacgcacagaagttccagggcagagtcaccttgaccgacgacacatctacagacacagcctacatggagctgagcagcctgagatctgaggacacggccgtgtattactgtgcgagggatctgggttaccttacttcggggaattattatgatgcttttgatatctggggccgagggacaatgatcaccgtctcctcagctagcaccaagggcccatcggtcttccccctggcgccctcctccaagagcacctctgggggcacagcggccctgggctgcctggtcaaggactacttccccgaaccggtgacggtgtcgtggaactcaggggccctgaccagcggcgtgcacaccttcccggctgtcctacagtcctcaggactctactccctcagcagcgtggtgaccgtgccctccagcagcctgggcacccagacctacatctgcaacgtgaatcacaagcccagcaacaccaaggtggacaagaaagttgagcccaaatcttgtgacaaaactcacacatgcccaccgtgcccagcacctgaactcctggggggaccgtcagtcttcctcttccccccaaaacccaaggacaccctcatgatctcccggacccctgaggtcacatgcgtggtggtggacgtgagccacgaagaccctgaggtcaagttcaactggtacgtggacggcgtggaggtgcataatgccaagacaaagccgcgggaggagcagtacaacagcacgtaccgtgtggtcagcgtcctcaccgtcctgcaccaggactggctgaatggcaaggagtacaagtgcaaggtctccaacaaagccctcccagcccccatcgagaaaaccatctccaaagccaaagggcagccccgagaaccacaggtgtacaccctgcccccatcccgggaggagatgaccaagaaccaggtcagcctgacctgcctggtcaaaggcttctatcccagcgacatcgccgtggagtgggagagcaatgggcagccggagaacaactacaagaccacgcctcccgtgctggactccgacggctccttcttcctctacagcaagctcaccgtggacaagagcaggtggcagcaggggaacgtcttctcatgctccgtgatgcatgaggctctgcacaaccactacacgcagaagagcctctccctgtctccgggtaaa

SEQ ID NO: 71 - protein, 455 aa, synthetic construct
QMQLVQSGAEVKKPGASVKVSCKVSGYPLSELSIHWVRQAPGKGLEWMGGFDSEDDETVYAQKFQGRVTLTDDTSTDTAYMELSSLRSEDTAVYYCARDLGYLTSGNYYDAFGIWGRGTMITVSSASTKGPSVFPLAPSSKSTSGGTAALGCLVKDYFPEPVTVSWNSGALTSGVHTFPAVLQSSGLYSLSSVVTVPSSSLGTQTYICNVNHKPSNTKVDKKVEPKSCDKTHTCPPCPAPELLGGPSVFLFPPKPKDTLMISRTPEVTCVVVDVSHEDPEVKFNWYVDGVEVHNAKTKPREEQYNSTYRVVSVLTVLHQDWLNGKEYKCKVSNKALPAPIEKTISKAKGQPREPQVYTLPPSREEMTKNQVSLTCLVKGFYPSDIAVEWESNGQPENNYKTTPPVLDSDGSFFLYSKLTVDKSRWQQGNVFSCSVMHEALHNHYTQKSLSLSPGK

SEQ ID NO: 72 - DNA, 1365 bp, synthetic construct
  source 1..1365: mol_type = other DNA
cagatgcagctggtacagtctggggctgaggtgaagaagcctggggcctcagtgaaggtctcctgcaaagtttccggttacccccttagtgagttatccattcactgggtgcgacaggctcctggaaaagggcttgagtggatggggggttttgattctgaagatgatgaaacagtctacgcacagaagttccagggcagagtcaccttgaccgacgacacatctacagacacagcctacatggagctgagcagcctgagatctgaggacacggccgtgtattactgtgcgagggatctgggttaccttacttcggggaattattatgatgcttttggtatctggggccgagggacaatgatcaccgtctcctcagctagcaccaagggcccatcggtcttccccctggcgccctcctccaagagcacctctgggggcacagcggccctgggctgcctggtcaaggactacttccccgaaccggtgacggtgtcgtggaactcaggggccctgaccagcggcgtgcacaccttcccggctgtcctacagtcctcaggactctactccctcagcagcgtggtgaccgtgccctccagcagcctgggcacccagacctacatctgcaacgtgaatcacaagcccagcaacaccaaggtggacaagaaagttgagcccaaatcttgtgacaaaactcacacatgcccaccgtgcccagcacctgaactcctggggggaccgtcagtcttcctcttccccccaaaacccaaggacaccctcatgatctcccggacccctgaggtcacatgcgtggtggtggacgtgagccacgaagaccctgaggtcaagttcaactggtacgtggacggcgtggaggtgcataatgccaagacaaagccgcgggaggagcagtacaacagcacgtaccgtgtggtcagcgtcctcaccgtcctgcaccaggactggctgaatggcaaggagtacaagtgcaaggtctccaacaaagccctcccagcccccatcgagaaaaccatctccaaagccaaagggcagccccgagaaccacaggtgtacaccctgcccccatcccgggaggagatgaccaagaaccaggtcagcctgacctgcctggtcaaaggcttctatcccagcgacatcgccgtggagtgggagagcaatgggcagccggagaacaactacaagaccacgcctcccgtgctggactccgacggctccttcttcctctacagcaagctcaccgtggacaagagcaggtggcagcaggggaacgtcttctcatgctccgtgatgcatgaggctctgcacaaccactacacgcagaagagcctctccctgtctccgggtaaa

SEQ ID NO: 73 - protein, 455 aa, synthetic construct
QMQLVQSGAEVKKPGASVKVSCKVSGYTLSELSIHWVRQAPGKGLEWMGGFDPEDDETVYAQKFQGRVTLTDDTSTDTAYMELSSLRSEDTAVYYCARDLGYLTSGNYYNAFGIWGRGTMITVSSASTKGPSVFPLAPSSKSTSGGTAALGCLVKDYFPEPVTVSWNSGALTSGVHTFPAVLQSSGLYSLSSVVTVPSSSLGTQTYICNVNHKPSNTKVDKKVEPKSCDKTHTCPPCPAPELLGGPSVFLFPPKPKDTLMISRTPEVTCVVVDVSHEDPEVKFNWYVDGVEVHNAKTKPREEQYNSTYRVVSVLTVLHQDWLNGKEYKCKVSNKALPAPIEKTISKAKGQPREPQVYTLPPSREEMTKNQVSLTCLVKGFYPSDIAVEWESNGQPENNYKTTPPVLDSDGSFFLYSKLTVDKSRWQQGNVFSCSVMHEALHNHYTQKSLSLSPGK

SEQ ID NO: 74 - DNA, 1365 bp, synthetic construct
  source 1..1365: mol_type = other DNA
cagatgcagctggtacagtctggggctgaggtgaagaagcctggggcctcagtgaaggtctcctgcaaagtttccggttacacccttagtgagttatccattcactgggtgcgacaggctcctggaaaagggcttgagtggatggggggttttgatcctgaagatgatgaaacagtctacgcacagaagttccagggcagagtcaccttgaccgacgacacatctacagacacagcctacatggagctgagcagcctgagatctgaggacacggccgtgtattactgtgcgagggatctgggttaccttacttcggggaattattataatgcttttggtatctggggccgagggacaatgatcaccgtctcctcagctagcaccaagggcccatcggtcttccccctggcgccctcctccaagagcacctctgggggcacagcggccctgggctgcctggtcaaggactacttccccgaaccggtgacggtgtcgtggaactcaggggccctgaccagcggcgtgcacaccttcccggctgtcctacagtcctcaggactctactccctcagcagcgtggtgaccgtgccctccagcagcctgggcacccagacctacatctgcaacgtgaatcacaagcccagcaacaccaaggtggacaagaaagttgagcccaaatcttgtgacaaaactcacacatgcccaccgtgcccagcacctgaactcctggggggaccgtcagtcttcctcttccccccaaaacccaaggacaccctcatgatctcccggacccctgaggtcacatgcgtggtggtggacgtgagccacgaagaccctgaggtcaagttcaactggtacgtggacggcgtggaggtgcataatgccaagacaaagccgcgggaggagcagtacaacagcacgtaccgtgtggtcagcgtcctcaccgtcctgcaccaggactggctgaatggcaaggagtacaagtgcaaggtctccaacaaagccctcccagcccccatcgagaaaaccatctccaaagccaaagggcagccccgagaaccacaggtgtacaccctgcccccatcccgggaggagatgaccaagaaccaggtcagcctgacctgcctggtcaaaggcttctatcccagcgacatcgccgtggagtgggagagcaatgggcagccggagaacaactacaagaccacgcctcccgtgctggactccgacggctccttcttcctctacagcaagctcaccgtggacaagagcaggtggcagcaggggaacgtcttctcatgctccgtgatgcatgaggctctgcacaaccactacacgcagaagagcctctccctgtctccgggtaaa

SEQ ID NO: 75 - protein, 455 aa, synthetic construct
QMQLVQSGAEVKKPGASVKVSCKVSGYTLSGLSIHWVRQAPGKGLEWMGGFDSEDDETVYAQKFQGRVTLTDDTSTDTAYMELSSLRSEDTAVYYCARDLGYLTSGNYYDAFDIWGRGTMITVSSASTKGPSVFPLAPSSKSTSGGTAALGCLVKDYFPEPVTVSWNSGALTSGVHTFPAVLQSSGLYSLSSVVTVPSSSLGTQTYICNVNHKPSNTKVDKKVEPKSCDKTHTCPPCPAPELLGGPSVFLFPPKPKDTLMISRTPEVTCVVVDVSHEDPEVKFNWYVDGVEVHNAKTKPREEQYNSTYRVVSVLTVLHQDWLNGKEYKCKVSNKALPAPIEKTISKAKGQPREPQVYTLPPSREEMTKNQVSLTCLVKGFYPSDIAVEWESNGQPENNYKTTPPVLDSDGSFFLYSKLTVDKSRWQQGNVFSCSVMHEALHNHYTQKSLSLSPGK

SEQ ID NO: 76 - DNA, 1365 bp, synthetic construct
  source 1..1365: mol_type = other DNA
cagatgcagctggtacagtctggggctgaggtgaagaagcctggggcctcagtgaaggtctcctgcaaagtttccggttacacccttagtgggttatccattcactgggtgcgacaggctcctggaaaagggcttgagtggatggggggttttgattctgaagatgatgaaacagtctacgcacagaagttccagggcagagtcaccttgaccgacgacacatctacagacacagcctacatggagctgagcagcctgagatctgaggacacggccgtgtattactgtgcgagggatctgggttaccttacttcggggaattattatgatgcttttgatatctggggccgagggacaatgatcaccgtctcctcagctagcaccaagggcccatcggtcttccccctggcgccctcctccaagagcacctctgggggcacagcggccctgggctgcctggtcaaggactacttccccgaaccggtgacggtgtcgtggaactcaggggccctgaccagcggcgtgcacaccttcccggctgtcctacagtcctcaggactctactccctcagcagcgtggtgaccgtgccctccagcagcctgggcacccagacctacatctgcaacgtgaatcacaagcccagcaacaccaaggtggacaagaaagttgagcccaaatcttgtgacaaaactcacacatgcccaccgtgcccagcacctgaactcctggggggaccgtcagtcttcctcttccccccaaaacccaaggacaccctcatgatctcccggacccctgaggtcacatgcgtggtggtggacgtgagccacgaagaccctgaggtcaagttcaactggtacgtggacggcgtggaggtgcataatgccaagacaaagccgcgggaggagcagtacaacagcacgtaccgtgtggtcagcgtcctcaccgtcctgcaccaggactggctgaatggcaaggagtacaagtgcaaggtctccaacaaagccctcccagcccccatcgagaaaaccatctccaaagccaaagggcagccccgagaaccacaggtgtacaccctgcccccatcccgggaggagatgaccaagaaccaggtcagcctgacctgcctggtcaaaggcttctatcccagcgacatcgccgtggagtgggagagcaatgggcagccggagaacaactacaagaccacgcctcccgtgctggactccgacggctccttcttcctctacagcaagctcaccgtggacaagagcaggtggcagcaggggaacgtcttctcatgctccgtgatgcatgaggctctgcacaaccactacacgcagaagagcctctccctgtctccgggtaaa

SEQ ID NO: 77 - protein, 455 aa, synthetic construct
QMQLVQSGAEVKKPGASVKVSCKVSGYTLSELSIHWVRQAPGKGLEWMGGFDSEDDETVYAQKFQGRVTLTDDTSTDTAYMELSSLRSEDTAVYYCARDLGYLTSGNYYDAFDFWGRGTMITVSSASTKGPSVFPLAPSSKSTSGGTAALGCLVKDYFPEPVTVSWNSGALTSGVHTFPAVLQSSGLYSLSSVVTVPSSSLGTQTYICNVNHKPSNTKVDKKVEPKSCDKTHTCPPCPAPELLGGPSVFLFPPKPKDTLMISRTPEVTCVVVDVSHEDPEVKFNWYVDGVEVHNAKTKPREEQYNSTYRVVSVLTVLHQDWLNGKEYKCKVSNKALPAPIEKTISKAKGQPREPQVYTLPPSREEMTKNQVSLTCLVKGFYPSDIAVEWESNGQPENNYKTTPPVLDSDGSFFLYSKLTVDKSRWQQGNVFSCSVMHEALHNHYTQKSLSLSPGK

SEQ ID NO: 78 - DNA, 1365 bp, synthetic construct
  source 1..1365: mol_type = other DNA
cagatgcagctggtacagtctggggctgaggtgaagaagcctggggcctcagtgaaggtctcctgcaaagtttccggttacacccttagtgagttatccattcactgggtgcgacaggctcctggaaaagggcttgagtggatggggggttttgattctgaagatgatgaaacagtctacgcacagaagttccagggcagagtcaccttgaccgacgacacatctacagacacagcctacatggagctgagcagcctgagatctgaggacacggccgtgtattactgtgcgagggatctgggttaccttacttcggggaattattatgatgcttttgatttctggggccgagggacaatgatcaccgtctcctcagctagcaccaagggcccatcggtcttccccctggcgccctcctccaagagcacctctgggggcacagcggccctgggctgcctggtcaaggactacttccccgaaccggtgacggtgtcgtggaactcaggggccctgaccagcggcgtgcacaccttcccggctgtcctacagtcctcaggactctactccctcagcagcgtggtgaccgtgccctccagcagcctgggcacccagacctacatctgcaacgtgaatcacaagcccagcaacaccaaggtggacaagaaagttgagcccaaatcttgtgacaaaactcacacatgcccaccgtgcccagcacctgaactcctggggggaccgtcagtcttcctcttccccccaaaacccaaggacaccctcatgatctcccggacccctgaggtcacatgcgtggtggtggacgtgagccacgaagaccctgaggtcaagttcaactggtacgtggacggcgtggaggtgcataatgccaagacaaagccgcgggaggagcagtacaacagcacgtaccgtgtggtcagcgtcctcaccgtcctgcaccaggactggctgaatggcaaggagtacaagtgcaaggtctccaacaaagccctcccagcccccatcgagaaaaccatctccaaagccaaagggcagccccgagaaccacaggtgtacaccctgcccccatcccgggaggagatgaccaagaaccaggtcagcctgacctgcctggtcaaaggcttctatcccagcgacatcgccgtggagtgggagagcaatgggcagccggagaacaactacaagaccacgcctcccgtgctggactccgacggctccttcttcctctacagcaagctcaccgtggacaagagcaggtggcagcaggggaacgtcttctcatgctccgtgatgcatgaggctctgcacaaccactacacgcagaagagcctctccctgtctccgggtaaa

SEQ ID NO: 79 - protein, 6 aa, synthetic construct
QDINRW

SEQ ID NO: 80 - DNA, 18 bp, synthetic construct
  source 1..18: mol_type = other DNA
caggatattaacaggtgg

SEQ ID NO: 81 - protein, 6 aa, synthetic construct
SQDINR

SEQ ID NO: 82 - DNA, 18 bp, synthetic construct
  source 1..18: mol_type = other DNA
agtcaggatattaacagg

SEQ ID NO: 83-86 - skipped (4 entries)

SEQ ID NO: 87 - protein, 9 aa, synthetic construct
QQTNNFPRT

SEQ ID NO: 88 - DNA, 27 bp, synthetic construct
  source 1..27: mol_type = other DNA
caacagactaacaatttccctcgaacc

SEQ ID NO: 89 - protein, 9 aa, synthetic construct
CQQTNNFPR

SEQ ID NO: 90 - DNA, 27 bp, synthetic construct
  source 1..27: mol_type = other DNA
tgtcaacagactaacaatttccctcga

SEQ ID NO: 91 - protein, 108 aa, synthetic construct
DIQMTQSPSSVSASVGDRVTITCRASQDINRWLAWYQQKPGKAPKLLIYAASRLQSGVPLRFSGSGSGTDFTLTINSLQPEDSATYYCQQTNNFPRTFGQGTRLEIKR

SEQ ID NO: 92 - DNA, 324 bp, synthetic construct
  source 1..324: mol_type = other DNA
gacatccagatgacccagtctccatcttccgtgtctgcatctgtgggagacagagtcaccatcacttgtcgggcgagtcaggatattaacaggtggttagcctggtatcaacagaaacctgggaaagcccctaagctcctgatctatgctgcatccagattgcaaagtggggtcccgttaagattcagcggcagtggatctgggacagatttcactctcactatcaacagcctgcagcccgaagattctgcaacttattactgtcaacagactaacaatttccctcgaaccttcggccaagggacacgactggagatcaaacgt

SEQ ID NO: 93 - DNA, 324 bp, synthetic construct
  source 1..324: mol_type = other DNA
gacatccagatgacccagtctccatcttccgtgtctgcatctgtgggagacagggtcaccatcacttgtcgggcgagtcaggatattaacaggtggttagcctggtatcaacagaaacctgggaaagcccctaagctcctgatctatgctgcatccagattgcaaagtggggtcccgttaagattcagcggcagtggatctgggacagatttcactctcactatcaacagcctgcagcccgaagattctgcaacttattactgtcaacagactaacaatttccctcgaaccttcggccaagggacacgactggagatcaaacgt

SEQ ID NO: 94 - protein, 214 aa, synthetic construct
DIQMTQSPSSVSASVGDRVTITCRASQDINRWLAWYQQKPGKAPKLLIYAASRLQSGVPLRFSGSGSGTDFTLTINSLQPEDSATYYCQQTNNFPRTFGQGTRLEIKRTVAAPSVFIFPPSDEQLKSGTASVVCLLNNFYPREAKVQWKVDNALQSGNSQESVTEQDSKDSTYSLSSTLTLSKADYEKHKVYACEVTHQGLSSPVTKSFNRGEC

SEQ ID NO: 95 - DNA, 642 bp, synthetic construct
  source 1..642: mol_type = other DNA
gacatccagatgacccagtctccatcttccgtgtctgcatctgtgggagacagagtcaccatcacttgtcgggcgagtcaggatattaacaggtggttagcctggtatcaacagaaacctgggaaagcccctaagctcctgatctatgctgcatccagattgcaaagtggggtcccgttaagattcagcggcagtggatctgggacagatttcactctcactatcaacagcctgcagcccgaagattctgcaacttattactgtcaacagactaacaatttccctcgaaccttcggccaagggacacgactggagatcaaacgtacggtggctgcaccatctgtcttcatcttcccgccatctgatgagcagttgaaatctggaactgcctctgttgtgtgcctgctgaataacttctatcccagagaggccaaagtacagtggaaggtggataacgccctccaatcgggtaactcccaggagagtgtcacagagcaggacagcaaggacagcacctacagcctcagcagcaccctgacgctgagcaaagcagactacgagaaacacaaagtctacgcctgcgaagtcacccatcagggcctgagctcgcccgtcacaaagagcttcaacaggggagagtgt

SEQ ID NO: 96 - DNA, 642 bp, synthetic construct
  source 1..642: mol_type = other DNA
gacatccagatgacccagtctccatcttccgtgtctgcatctgtgggagacagggtcaccatcacttgtcgggcgagtcaggatattaacaggtggttagcctggtatcaacagaaacctgggaaagcccctaagctcctgatctatgctgcatccagattgcaaagtggggtcccgttaagattcagcggcagtggatctgggacagatttcactctcactatcaacagcctgcagcccgaagattctgcaacttattactgtcaacagactaacaatttccctcgaaccttcggccaagggacacgactggagatcaaacgtacggtggctgcaccatctgtcttcatcttcccgccatctgatgagcagttgaaatctggaactgcctctgttgtgtgcctgctgaataacttctatcccagagaggccaaagtacagtggaaggtggataacgccctccaatcgggtaactcccaggagagtgtcacagagcaggacagcaaggacagcacctacagcctcagcagcaccctgacgctgagcaaagcagactacgagaaacacaaagtctacgcctgcgaagtcacccatcagggcctgagctcgcccgtcacaaagagcttcaacaggggagagtgt

SEQ ID NO: 97 - RNA, 29 nt, synthetic construct
  source 1..29: mol_type = other RNA
cgtgacctcaaacgcctagctgccaatga

SEQ ID NO: 98 - RNA, 29 nt, synthetic construct
  source 1..29: mol_type = other RNA
agcctcgaccgtctcctactgcaccagaa

SEQ ID NO: 99 - RNA, 19 nt, synthetic construct
  source 1..19: mol_type = other RNA
ccacccagatcgcggtata

SEQ ID NO: 100 - RNA, 19 nt, synthetic construct
  source 1..19: mol_type = other RNA
gcatcttcctgcacggcaa

SEQ ID NO: 101 - RNA, 19 nt, synthetic construct
  source 1..19: mol_type = other RNA
cgaatgtgctggcccgaat

SEQ ID NO: 102 - RNA, 19 nt, synthetic construct
  source 1..19: mol_type = other RNA
gagcccaaggtgacgacaa

SEQ ID NO: 103 - RNA, 19 nt, synthetic construct
  source 1..19: mol_type = other RNA
cggcaggcaatgcgctgaa

SEQ ID NO: 104 - RNA, 19 nt, synthetic construct
  source 1..19: mol_type = other RNA
caacaatctatcagcgctg

SEQ ID NO: 105 - RNA, 19 nt, synthetic construct
  source 1..19: mol_type = other RNA
aggccaggctgttcacgca

SEQ ID NO: 106 - RNA, 19 nt, synthetic construct
  source 1..19: mol_type = other RNA
aaatatcggacgacgtgga

SEQ ID NO: 107 - DNA, 19 bp, synthetic construct
  source 1..19: mol_type = other DNA
gcatcttcctgcacggcaa

SEQ ID NO: 108 - DNA, 19 bp, synthetic construct
  source 1..19: mol_type = other DNA
cgaatgtgctggcccgaat

SEQ ID NO: 109 - DNA, 19 bp, synthetic construct
  source 1..19: mol_type = other DNA
cggcaggcaatgcgctgaa

SEQ ID NO: 110 - DNA, 19 bp, synthetic construct
  source 1..19: mol_type = other DNA
aggccaggctgttcacgca

SEQ ID NO: 111 - protein, 40 aa, synthetic construct
RIYKGVIQAIQKSDEGHPFRAYLESEVAISEELVQKYSNS